European Patent Specification EP 2 988 774 B1, published June 5, 2024. Title: TOLERIZING TREATMENTS FOR AUTOIMMUNE DISEASE. Applicant: NUSSENBLATT, RICHARD LIU, BAOYING WEI, LAI RABBANI, ELAZAR DONEGAN, JAMES J. Application 13/871,730. The sequence listing filed with the application follows.

SEQUENCE LISTING (2 sequences)

SEQ ID NO: 1 - protein, 20 aa, Artificial Sequence
  Description of Artificial Sequence: Synthetic peptide
GEPIPVTVDVTNNTEKTVKK

SEQ ID NO: 2 - protein, 14 aa, Artificial Sequence
  Description of Artificial Sequence: Synthetic peptide
ALNEDLSSWTAADT